European Patent Application EP 4 219 758 A1, published August 2, 2023. Title: Method for detecting off-type of Brassica Oleracea plant. Applicant: Sakata Seed Corporation. The sequence listing filed with the application follows.

SEQUENCE LISTING (27 sequences)

SEQ ID NO: 1 - DNA, 22 bp, synthetic construct
  source 1..22: mol_type = other DNA; note = primer
ctggcaaatgtaagccctttct

SEQ ID NO: 2 - DNA, 26 bp, synthetic construct
  source 1..26: mol_type = other DNA; note = primer
cttgtcttattacagcagatgcattc

SEQ ID NO: 3 - DNA, 23 bp, synthetic construct
  source 1..23: mol_type = other DNA; note = primer
cgccattgctttctctctactct

SEQ ID NO: 4 - DNA, 22 bp, synthetic construct
  source 1..22: mol_type = other DNA; note = primer
gaagaggaaggactcgaggaag

SEQ ID NO: 5 - DNA, 21 bp, synthetic construct
  source 1..21: mol_type = other DNA; note = primer
cttaggattcgggttcgtttg

SEQ ID NO: 6 - DNA, 24 bp, synthetic construct
  source 1..24: mol_type = other DNA; note = primer
gccgtaagatttcaaagagacttc

SEQ ID NO: 7 - DNA, 21 bp, synthetic construct
  source 1..21: mol_type = other DNA; note = primer
cgtctcttgtggtggttgaag

SEQ ID NO: 8 - DNA, 23 bp, synthetic construct
  source 1..23: mol_type = other DNA; note = primer
tcaacttcatctgcttggtaatg

SEQ ID NO: 9 - DNA, 21 bp, synthetic construct
  source 1..21: mol_type = other DNA; note = primer
agcacatcatcccccatactt

SEQ ID NO: 10 - DNA, 23 bp, synthetic construct
  source 1..23: mol_type = other DNA; note = primer
cagtctctctctccttgatgacg

SEQ ID NO: 11 - DNA, 22 bp, synthetic construct
  source 1..22: mol_type = other DNA; note = primer
aggaagaggaaattgtcattcg

SEQ ID NO: 12 - DNA, 20 bp, synthetic construct
  source 1..20: mol_type = other DNA; note = primer
gtgaccgttgcagcagataa

SEQ ID NO: 13 - DNA, 26 bp, synthetic construct
  source 1..26: mol_type = other DNA; note = primer
aagaaattagccacaagtcgtaaata

SEQ ID NO: 14 - DNA, 25 bp, synthetic construct
  source 1..25: mol_type = other DNA; note = primer
acgtgaatgatggatatttgatctc

SEQ ID NO: 15 - DNA, 24 bp, synthetic construct
  source 1..24: mol_type = other DNA; note = primer
aaagctcgtgaagcaaatactacc

SEQ ID NO: 16 - DNA, 23 bp, synthetic construct
  source 1..23: mol_type = other DNA; note = primer
gaagcataccaggagggaaataa

SEQ ID NO: 17 - DNA, 20 bp, synthetic construct
  source 1..20: mol_type = other DNA; note = primer
gccatcgcgaatcaaagata

SEQ ID NO: 18 - DNA, 23 bp, synthetic construct
  source 1..23: mol_type = other DNA; note = primer
atttggtattttgcaggctacag

SEQ ID NO: 19 - DNA, 30 bp, synthetic construct
  source 1..30: mol_type = other DNA; note = probe
cacttgtaaaacatgggtttgatcaaaaga

SEQ ID NO: 20 - DNA, 24 bp, synthetic construct
  source 1..24: mol_type = other DNA; note = probe
tcctctacttccaccccatctgcc

SEQ ID NO: 21 - DNA, 25 bp, synthetic construct
  source 1..25: mol_type = other DNA; note = probe
ccgatctgaaaagggagctaacgac

SEQ ID NO: 22 - DNA, 25 bp, synthetic construct
  source 1..25: mol_type = other DNA; note = probe
ttgcagcaaggagcttagaccacag

SEQ ID NO: 23 - DNA, 25 bp, synthetic construct
  source 1..25: mol_type = other DNA; note = probe
tctcgagaaatctcatcgctgcttg

SEQ ID NO: 24 - DNA, 25 bp, synthetic construct
  source 1..25: mol_type = other DNA; note = probe
ttctcagagctgttccctcctccac

SEQ ID NO: 25 - DNA, 27 bp, synthetic construct
  source 1..27: mol_type = other DNA; note = probe
ttgcaccaccgttaccttttaacacaa

SEQ ID NO: 26 - DNA, 26 bp, synthetic construct
  source 1..26: mol_type = other DNA; note = probe
tgttttgtttggtgggcaaatctctt

SEQ ID NO: 27 - DNA, 25 bp, synthetic construct
  source 1..25: mol_type = other DNA; note = probe
tggagatcttccacctcatcttgga